European Patent Specification EP 3 957 750 B1, published January 29, 2025. Title: Preserving Genomic Connectivity Information In Fragmented Genomic DNA Samples. Applicant: Illumina, Inc. The sequence listing filed with the application follows.

SEQUENCE LISTING (3 sequences)

SEQ ID NO: 1 - DNA, 35 bp, Artificial Sequence
  Sequencing Read A and B
cttaaaaagagcatgttttaccttttgtaaattat

SEQ ID NO: 2 - DNA, 16 bp, Artificial Sequence
  Sequencing Read C
gtaaattatatctcaa

SEQ ID NO: 3 - DNA, 44 bp, Artificial Sequence
  Target Sequence Fragment
tacttaaaaagagcatgttttacattttgtaaattatatctcaa